European Patent Application EP 4 692 128 A1, published February 11, 2026. Title: FUSION PROTEIN, CORRESPONDING NUCLEIC ACID, IN-VITRO SYNTHESIS SYSTEM, AND PREPARATION METHOD. Applicant: KANGMA-HEATHCODE (SHANGHAI) BIOTECH CO., LTD. The sequence listing filed with the application follows.

SEQUENCE LISTING (66 sequences)

SEQ ID NO: 1 - protein, 389 aa, synthetic construct
GADDVVDSSKSFVMENFSSYHGTKPGYVDSIQKGIQKPKSGTQGNYDDDWKGFYSTDNKYDAAGYSVDNENPLSGKAGGVVKVTYPGLTKVLALKVDNAETIKKELGLSLTEPLMEQVGTEEFIKRFGDGASRVVLSLPFAEGSSSVEYINNWEQAKALSVELEINFETRGKRGQDAMYEYMAQACAGNRVRRSVGSSLSCINLDWDVIRDKTKTKIESLKEHGPIKNKMSESPNKTVSEEKAKQYLEEFHQTALEHPELSELKTVTGTNPVFAGANYAAWAVNVAQVIDSETADNLEKTTAALSILPGIGSVMGIADGAVHHNTEEIVAQSIALSSLMVAQAIPLVGELVDIGFAAYNFVESIINLFQVVHNSYNRPAYSPGHKTQPF

SEQ ID NO: 2 - protein, 195 aa, synthetic construct
SVGSSLSCINLDWDVIRDKTKTKIESLKEHGPIKNKMSESPNKTVSEEKAKQYLEEFHQTALEHPELSELKTVTGTNPVFAGANYAAWAVNVAQVIDSETADNLEKTTAALSILPGIGSVMGIADGAVHHNTEEIVAQSIALSSLMVAQAIPLVGELVDIGFAAYNFVESIINLFQVVHNSYNRPAYSPGHKTQP

SEQ ID NO: 3 - protein, 193 aa, synthetic construct
GADDVVDSSKSFVMENFSSYHGTKPGYVDSIQKGIQKPKSGTQGNYDDDWKGFYSTDNKYDAAGYSVDNENPLSGKAGGVVKVTYPGLTKVLALKVDNAETIKKELGLSLTEPLMEQVGTEEFIKRFGDGASRVVLSLPFAEGSSSVEYINNWEQAKALSVELEINFETRGKRGQDAMYEYMAQACAGNRVRR

SEQ ID NO: 4 - protein, 347 aa, synthetic construct
PEGGSLAALTAHQACHLPLETFTRHRQPRGWEQLEQCGYPVQRLVALYLAARLSWNQVDQVIRNALASPGSGGDLGEAIREQPEQARLALTLAAAESERFVRQGTGNDEAGAANGPADSGDALLERNYPTGAEFLGDGGDVSFSTRGTQNWTVERLLQAHRQLEERGYVFVGYHGTFLEAAQSIVFGGVRARSQDLDAIWRGFYIAGDPALAYGYAQDQEPDARGRIRNGALLRVYVPRSSLPGFYRTSLTLAAPEAAGEVERLIGHPLPLRLDAITGPEEEGGRLETILGWPLAERTVVIPSAIPTDPRNVGGDLDPSSIPDKEQAISALPDYASQPGKPPREDLK

SEQ ID NO: 5 - protein, 107 aa, synthetic construct
PEGGSLAALTAHQACHLPLETFTRHRQPRGWEQLEQCGYPVQRLVALYLAARLSWNQVDQVIRNALASPGSGGDLGEAIREQPEQARLALTLAAAESERFVRQGTGN

SEQ ID NO: 6 - protein, 215 aa, synthetic construct
EFLGDGGDISFSTRGTQNWTVERLLQAHRQLEERGYVFVGYHGTFLEAAQSIVFGGVRARSQDLDAIWRGFYIAGDPALAYGYAQDQEPDARGRIRNGALLRVYVPRSSLPGFYRTGLTLAAPEAAGEVERLIGHPLPLRLDAITGPEEEGGRLETILGWPLAERTVVIPSAIPTDPRNVGGDLDPSSIPDKEQAISALPDYASQPGKPPREDLK

SEQ ID NO: 7 - protein, 634 aa, synthetic construct
VEDELNIFDECRSPCSLTPEPGKPIQSKLSIPSDVVLDEGVLYYSMTINDEQNDIKDEDKGESIITIGEFATVRATRHYVNQDAPFGVIHLDITTENGTKTYSYNRKEGEFAINWLVPIGEDSPASIKISVDELDQQRNIIEVPKLYSIDLDNQTLEQWKTQGNVSFSVTRPEHNIAISWPSVSYKAAQKEGSRHKRWAHWHTGLALCWLVPMDAIYNYITQQNCTLGDNWFGGSYETVAGTPKVITVKQGIEQKPVEQRIHFSKGNAMSALAAHRVCGVPLETLARSRKPRDLTDDLSCAYQAQNIVSLFVATRILFSHLDSVFTLNLDEQEPEVAERLSDLRRINENNPGMVTQVLTVARQIYNDYVTHHPGLTPEQTSAGAQAADILSLFCPDADKSCVASNNDQANINIESRSGRSYLPENRAVITPQGVTNWTYQELEATHQALTREGYVFVGYHGTNHVAAQTIVNRIAPVPRGNNTENEEKWGGLYVATHAEVAHGYARIKEGTGEYGLPTRAERDARGVMLRVYIPRASLERFYRTNTPLENAEEHITQVIGHSLPLRNEAFTGPESAGGEDETVIGWDMAIHAVAIPSTIPGNAYEELAIDEEAVAKEQSISTKPPYKERKDELK

SEQ ID NO: 8 - protein, 426 aa, synthetic construct
VEDELNIFDECRSPCSLTPEPGKPIQSKLSIPSDVVLDEGVLYYSMTINDEQNDIKDEDKGESIITIGEFATVRATRHYVNQDAPFGVIHLDITTENGTKTYSYNRKEGEFAINWLVPIGEDSPASIKISVDELDQQRNIIEVPKLYSIDLDNQTLEQWKTQGNVSFSVTRPEHNIAISWPSVSYKAAQKEGSRHKRWAHWHTGLALCWLVPMDAIYNYITQQNCTLGDNWFGGSYETVAGTPKVITVKQGIEQKPVEQRIHFSKGNAMSALAAHRVCGVPLETLARSRKPRDLTDDLSCAYQAQNIVSLFVATRILFSHLDSVFTLNLDEQEPEVAERLSDLRRINENNPGMVTQVLTVARQIYNDYVTHHPGLTPEQTSAGAQAADILSLFCPDADKSCVASNNDQANINIESRSGRSYLPENR

SEQ ID NO: 9 - protein, 426 aa, synthetic construct; identical to SEQ ID NO: 8

SEQ ID NO: 10 - protein, 5 aa, synthetic construct
GGGGS

SEQ ID NO: 11 - protein, 7 aa, synthetic construct
EASGGPE

SEQ ID NO: 12 - protein, 60 aa, synthetic construct
GGSSGSGSGSTGTSSSGTGTSAGTTGTSASTSGSGSGGGGGSGGGGSAGGTATAGASSGS

SEQ ID NO: 13 - protein, 36 aa, synthetic construct
GAGAGSGAGAGSGAGAGSGAGAGSGAGAGSGAGAGS

SEQ ID NO: 14 - protein, 5 aa, synthetic construct
GGGGS

SEQ ID NO: 15 - skipped

SEQ ID NO: 16 - protein, 12 aa, synthetic construct
KESGSVSSEQLA

SEQ ID NO: 17 - protein, 448 aa, synthetic construct
EVQLVQSGAEVKKPGASVKVSCKASGYRFTNYWIHWVRQAPGQGLEWIGGINPGNNYATYRRKFQGRVTMTADTSTSTVYMELSSLRSEDTAVYYCTREGYGNYGAWFAYWGQGTLVTVSSASTKGPSVFPLAPCSRSTSESTAALGCLVKDYFPEPVTVSWNSGALTSGVHTFPAVLQSSGLYSLSSVVTVPSSSLGTKTYTCNVDHKPSNTKVDKRVESKYGPPCPPCPAPEFLGGPSVFLFPPKPKDTLMISRTPEVTCVVVDVSQEDPEVQFNWYVDGVEVHNAKTKPREEQFNSTYRVVSVLTVLHQDWLNGKEYKCKVSNKGLPSSIEKTISKAKGQPREPQVYTLPPSQEEMTKNQVSLTCLVKGFYPSDIAVEWESNGQPENNYKTTPPVLDSDGSFFLYSRLTVDKSRWQEGNVFSCSVMHEALHNHYTQKSLSLSLGK

SEQ ID NO: 18 - protein, 11 aa, synthetic construct
EGKSSGSGSES

SEQ ID NO: 19 - protein, 9 aa, synthetic construct
GSAPAPAGS

SEQ ID NO: 20 - protein, 5 aa, synthetic construct
GGGGS

SEQ ID NO: 21 - skipped

SEQ ID NO: 22 - protein, 8 aa, synthetic construct
GGSGGGGS

SEQ ID NO: 23 - protein, 22 aa, synthetic construct
GGSHHGHKTQPFGGGGSGGGGS

SEQ ID NO: 24 - protein, 19 aa, synthetic construct
GGSHHTQPFGGGGSGGGGS

SEQ ID NO: 25 - protein, 15 aa, synthetic construct
GGSHHQPFEASGGPE

SEQ ID NO: 26 - protein, 12 aa, synthetic construct
GGSHHEASGGPE

SEQ ID NO: 27 - protein, 9 aa, synthetic construct
GGSHHGGPE

SEQ ID NO: 28 - protein, 5 aa, synthetic construct
GGGGS

SEQ ID NO: 29 - protein, 9 aa, synthetic construct
SHGGSLGGS

SEQ ID NO: 30 - protein, 8 aa, synthetic construct
GGSHHGGS

SEQ ID NO: 31 - protein, 12 aa, synthetic construct
KESGSVSSEQLA

SEQ ID NO: 32 - protein, 214 aa, synthetic construct
DIQMTQSPSSLSASVGDRVTITCRASQDVNTAVAWYQQKPGKAPKLLIYSASFLYSGVPSRFSGSRSGTDFTLTISSLQPEDFATYYCQQHYTTPPTFGQGTKVEIKRTVAAPSVFIFPPSDEQLKSGTASVVCLLNNFYPREAKVQWKVDNALQSGNSQESVTEQDSKDSTYSLSSTLTLSKADYEKHKVYACEVTHQGLSSPVTKSFNRGEC

SEQ ID NO: 33 - protein, 120 aa, synthetic construct [sequence omitted]

SEQ ID NO: 34 - protein, 105 aa, synthetic construct
ASTKGPSVFPLAPSSKSTSGGTAALGCLVKDYFPEPVTVSWNSGALTSGVHTFPAVLQSSGLYSLSSVVTVPSSSLGTQTYICNVNHKPSNTKVDKKVEPKSCDK

SEQ ID NO: 35 - protein, 118 aa, synthetic construct
EVQLVESGGGSDIQMTQSPSSLSASVGDRVTITCRASQDVNTAVAWYQQKPGKAPKLLIYSASFLYSGVPSRFSGSRSGTDFTLTISSLQPEDFATYYCQQHYTTPPTFGQGTKVEIK

SEQ ID NO: 36 - protein, 225 aa, synthetic construct
EVQLVESGGGLVQPGGSLRLSCAASGFNIKDTYIHWVRQAPGKGLEWVARIYPTNGYTRYADSVKGRFTISADTSKNTAYLQMNSLRAEDTAVYYCSRWGGDGFYAMDYWGQGTLVTVSSASTKGPSVFPLAPSSKSTSGGTAALGCLVKDYFPEPVTVSWNSGALTSGVHTFPAVLQSSGLYSLSSVVTVPSSSLGTQTYICNVNHKPSNTKVDKKVEPKSCDK

SEQ ID NO: 37 - protein, 107 aa, synthetic construct
GQPREPQVYTLPPSREEMTKNQVSLTCLVKGFYPSDIAVEWESNGQPENNYKTTPPVLDSDGSFFLYSKLTVDKSRWQQGNVFSCSVMHEALHNHYTQKSLSLSPGK

SEQ ID NO: 38 - protein, 140 aa, synthetic construct
SDVQSSLTGTWYNELNSKMELTANKDGTLTGKYLSKVGDVYVPYPLSGRYNLQPPAGQGVALGWAVSWENSKIHSATTWSGQFFSESSPVILTQWLLSSSTARGDVWESTLVGNDSFTKTAPTEQQIAHAQLHCRAPRLK

SEQ ID NO: 39 - DNA, 46 bp, synthetic construct
  source 1..46: mol_type = other DNA
ctggtggtggtggttctgacatccaaatgacccaatctccatcttc

SEQ ID NO: 40 - DNA, 46 bp, synthetic construct
  source 1..46: mol_type = other DNA
gtggtggtgagaaccacccttgtcacaagactttggttcaaccttc

SEQ ID NO: 41 - DNA, 42 bp, synthetic construct
  source 1..42: mol_type = other DNA
gaaccaaagtcttgtgacaagggtggttctcaccaccaccac

SEQ ID NO: 42 - DNA, 44 bp, synthetic construct
  source 1..44: mol_type = other DNA
ggagattgggtcatttggatgtcagaaccaccaccaccagaacc

SEQ ID NO: 43 - skipped

SEQ ID NO: 44 - protein, 19 aa, synthetic construct
GSAEAAAKEAAAKAGGGGS

SEQ ID NO: 45 - protein, 60 aa, synthetic construct; identical to SEQ ID NO: 12

SEQ ID NO: 46 - protein, 238 aa, synthetic construct
VSKGEELFTGVVPILVELDGDVNGHKFSVRGEGEGDATNGKLTLKFICTTGKLPVPWPTLVTTLTYGVQCFSRYPDHMKQHDFFKSAMPEGYVQERTISFKDDGTYKTRAEVKFEGDTLVNRIELKGIDFKEDGNILGHKLEYNFNSHNVYITADKQKNGIKANFKIRHNVEDGSVQLADHYQQNTPIGDGPVLLPDNHYLSTQSKLSKDPNEKRDHMVLLEFVTAAGITLGMDELYK

SEQ ID NO: 47 - protein, 18 aa, synthetic construct
GSTSGSGKPGSGEGSTKG

SEQ ID NO: 48 - protein, 12 aa, synthetic construct
GSAGSAAGSGEF

SEQ ID NO: 49 - protein, 12 aa, synthetic construct
GSAPAPAGGGGS

SEQ ID NO: 50 - protein, 12 aa, synthetic construct
KESGSVSSEQLA

SEQ ID NO: 51 - protein, 10 aa, synthetic construct
CPPCPAPELL

SEQ ID NO: 52 - protein, 117 aa, synthetic construct
EVQLQESGGGLVQPGGSLRLSCAASGFIFSNDAMTWVRQAPGKGLEWVSSINWSGTHTNYADSVKGRFTISRDNAKRTLYLQMNSLKDEDTALYYCVTGYGVTKTPTGQGTQVTVSS

SEQ ID NO: 53 - protein, 118 aa, synthetic construct
EVQLVESGGGLVQAGGSLRLSCAASGITFSINTMGWYRQAPGKQRELVALISSIGDTYYADSVKGRFTISRDNAKNTVYLQMNSLKPEDTAVYYCKRFRTAAQGTDYWGQGTQVTVSS

SEQ ID NO: 54 - protein, 113 aa, synthetic construct
DVQVTQSPSSLSASVGDRVTITCRSSQSLANSYGNTFLSWYLHKPGKAPQLLIYGISNRFSGVPDRFSGSGSGTDFTLTISSLQPEDFATYYCLQGTHQPYTFGQGTKVEIKR

SEQ ID NO: 55 - protein, 121 aa, synthetic construct
EVQLVQSGAEVKKPGASVKVSCKASGYRFTNYWIHWVRQAPGQGLEWIGGINPGNNYATYRRKFQGRVTMTADTSTSTVYMELSSLRSEDTAVYYCTREGYGNYGAWFAYWGQGTLVTVSS

SEQ ID NO: 56 - protein, 219 aa, synthetic construct
DVQVTQSPSSLSASVGDRVTITCRSSQSLANSYGNTFLSWYLHKPGKAPQLLIYGISNRFSGVPDRFSGSGSGTDFTLTISSLQPEDFATYYCLQGTHQPYTFGQGTKVEIKRTVAAPSVFIFPPSDEQLKSGTASVVCLLNNFYPREAKVQWKVDNALQSGNSQESVTEQDSKDSTYSLSSTLTLSKADYEKHKVYACEVTHQGLSSPVTKSFNRGEC

SEQ ID NO: 57 - protein, 100 aa, synthetic construct
ASTKGPSVFPLAPCSRSTSESTAALGCLVKDYFPEPVTVSWNSGALTSGVHTFPAVLQSSGLYSLSSVVTVPSSSLGTKTYTCNVDHKPSNTKVDKRVES

SEQ ID NO: 58 - protein, 8 aa, synthetic construct
HHHHHHHH

SEQ ID NO: 59 - protein, 422 aa, synthetic construct
MTMGEVEKKPRRRFVGIKKAAEESDPSGSTTELVKKIKPKTNIRHAINQIPPELLNDEELNAAIKLLPSNYNFEIHKTVWNIRKHKAKRVAIQMPEGLLIYSLVISDILEQFCQCEIVVMGDVSYGACCIDDYTARSLDCDFIVHYAHSCLVPIDITTIKVLYIFVTINIDETHLIKTLQKNFPRGSRIAAFGTIQFNPTIHSMKDKLLQSEEHMLYIIPPQIKPLSKGEVLGCTSERLNKEQIDAMVYVGDGRFHLESAMIHNPEIPAFRYDPYNRRFTRERYDQKQLVEVRASAIDKARSSKKVGLILGALGRQGNLATVENLETKLKASGRTVVKIILSEIFPQKLAMFDDIDAFVQVACPRLSIDWGYAFNKPLLTPYETNVMLENDRMFNEKYYPMDYYHINGYGRGKVPNHDDVTI

SEQ ID NO: 60 - protein, 587 aa, synthetic construct
MNDSVLVAPSLSTAQTEDTFEFQSYGETEHSRSYLGSDVTKDNLVELVSAYYSVPELIQYFEEHPQYKKITLQFPDELVLDSSIVVQLMQQELVKAEDETSQSFNTIDTDEVLHNEKSCGNCSGCDCSSKIDKTETKRKVWILADTSYSSCCVDEVASEHVKGDIVVHFGDACMNAVQKLPVVYSLGRPVLDLDLVVSQFKLKYAAKDQKICLMADAPHSMHMKSIYDILHDKEGYKNVVYSDINQDMLQSDTHIVGYNNAVEHDERLRKCVTCGNRNIYAEVDVSELNEYDLFHVTIPKDPHLLYLTTKFQSVTLYDPSSGMLNEGPFPSMMKRYKFMHMARTAGTIGILVNTLSLRNTKETMNKLTKLLKENGKKHYLFVVGKPNVAKLANFEPIDIWCILGCGQGGIVLDQYNEFYKPIITPYELLMALSDEVTWTGQWITDFKSIINQIENEVNDSDDMEQDILSSGTECRSDEDEAPEFNAVTGKYVSTSRPLRQIARLEIETPVEEVRASDSTELVKQFSQTVAIRNTVSTSAAFLQTRHWTGLGSDYKDDEDGEEDGATVEEGTAGVARSYQFDELNKKT

SEQ ID NO: 61 - protein, 428 aa, synthetic construct
MAEELLNKHDPKLAYVVKYNHDSPNPRELASPLEMKRVARPLRHIHYVPVKSLIFYSKNHPPQFSYETKIKTPISKDVISVQVEYVGLNPVDLKIFNSYTRHMNYEVGIGREYYGKISEVGSNLADTWSVGDEVCGTFWHPNLGKGTCESTILVDPKVDVVLPKPVNISTQQAASTFYCLGAAFNILDKLDQEGKLNQSSNILINGASTMTGIFALQLLKFHYRILNRIVLISSTSGMNFIKSNLPELVDELLFIDYAATNGKIYKPLSDLVASNELVEYNNETGNFITQPFGQGSFNLVLDFIGGYDIIGHSSSILSKDATYITTVGDNKSNYKKDTFNSWGTASSNIRKLFGQVLWSFDYQMFYFDPNAKLATNEWPKKCHELIESEVVKFIPVDRVYDWKEHQKAFSYLQTGRAHGKVVLKVEKF

SEQ ID NO: 62 - protein, 162 aa, synthetic construct
MQRSFYEILGIESDASNIEIKRAYRAMLLETHPDKSGLNYNSNGNNTSSHSVTDIQEAYQTLIDQDLRKKYDEELAESFKKLGFHNAGDGLDLFSLDLFDYSGDEQSFSMNCPRCQITDGFQLTEDALEEHAIDYEGGGYFVLVQCSACSLWLKVLFDVMEE

SEQ ID NO: 63 - protein, 298 aa, synthetic construct
MLYFIGLGLSYETDITVRGLNAIKQCSRVYLEHYTSILMTASLEELEEFYGKKVTLADRELVESGAEELLRDADKEDVAFLVVGDVFGATTHTDLVLRAKQRNIPVEVIHNASVMNAVGSCGLQLYNFGQTISMVFFTDSWRPDSWYDKIWENRKIGLHTLVLLDIKVKEQSIENMARGRLIYEPPRYMSIAQCCEQLLEIEETRGTEAYTPDTPCVAISRLGSASQTFKAGTIKELAEYDSGEPLHSLVILGRQTHELEIEYLLEFCDDREKFKQDVASDQEYFKPPAWVPPPEDED

SEQ ID NO: 64 - protein, 696 aa, synthetic construct
MKFVALISGGKDSNYNILHCLKQDHELIAFANLHPENEDEQELDSFMFQTVGHDLIRWYPECSGVPLYRQALHKNGSKNIALNYTETKDDEIEDLYKLLRKIQLDSPDLEAVSVGAILSSYQRTRVEDVCSRLGLTTLSYLWQRDQRELMQEMCSMSKDTIVTTDDCDNVGKLDARIIKVAAIGLNQNHLGKSLPEILPTMLKLNSLYDVHICGEGGEFETMVLDTPFFKHGHLQLNSINDVTDTSNDGVFAATFNVEYVPEALSPTKLEKELEKLPVPAVLNEKWYEMYLRLMTIDLKKLNNCPNHHNVSPSVPVSINEVGKLLYISNIAPSKGESLKEKCLDVFSQLTSILSSRSIFACQILSSSLLLSDMNNFQEVNSYYNEYFNVTKIGPLPPARACVESSFLKHPVQLSVVVDLSADCVPTDNGIILNRSKDGLHVQGRSYWCPCNIGPYSQATWNQSDRNKVTYISGQIGLEPSSMKLWGDTTLLENPDIAEVVLSLRNYFTLSETVNSSIPLTMVCYISQSYVLPAVRSAWSLFAKELAEESELWFDQEPVGVDSLVIVKVSNLPKNALCEWTGMNCQNLAIEDDYDEDDLAAQIHMNLTLKSQTDIELPNYAHDVIISENGFKRHFITLFLDSHEQLILTLSECKNAQITLFFSKDYAVPEYTHVEYIPVEQVYDKSSPRAYGLVIKY

SEQ ID NO: 65 - protein, 419 aa, synthetic construct
MAQQSLQKHPHDEDAEYDSNIGIAYHLRGATKLEVKSFCRMEETAADKRVTTRLPPCCLCILREKFIIVGTYLLHKDSGNRTGSIEVYDKELNLLSSIKTYGAILDLKLNPFDDTLLATAHSTGNMILWTISVDDDNSSIDIKLLNNLQVFDPTCLITSLQFSPLLDNLVLLTTTNGDFATVDIIHGEICFIEEVEPSYFDSSTINYIEVPNADIKVINVQNDHEQIFHFKHSLECWTGEFGCLAPLKDVVFTGGDDSAIAAHDLNSGKKIWSNSKIHQAGVTAIKAARETFRGNKPTSLITGSYDDHIRSFDLRMLSETTIYPGTDVPVVNKWEDNLQGGVWRFSEAPTNDGLSNNRLMVCCMYNGAKVVNVQNDHFVTEQFIKEGHESMCYGGDWSKETVATCSFYDKSLQLWKSPN

SEQ ID NO: 66 - protein, 842 aa, synthetic construct
MVAFTVDQIRSLMDKVTNVRNMSVIAHVDHGKSTLTDSLVQRAGIISAAKAGEARFTDTRKDEQERGITIKSTAISLFSEMSDDDVKDIKQKTDGNAFLINLIDSPGHVDFSSEVTAALRVTDGALVVVDTVEGVCVQTETVLRQSLAERIKPVVVINKVDRALLELQVSKEDLYQSFSRTVESVNVIISTYADEVLGDVQVYPQRGTVAFGSGLHGWAFTVRQFANRYSKKFGVDREKMMDRLWGDSYFNPKTKKWTNKERDADGKPLERAFNMFVLDPIFRLFAAIMNFKKEEIPVLLEKLEINLKGDEKELEGKNLLKVVMRKFLPAADALLEMIILHLPSPVTAQNYRAEQLYEGPSDDPACIAIKNCDPKSDLMLYVSKMVPTSDKGRFYAFGRVFAGTVKSGQKVRIQGPNFIPGKKEDLFIKAIQRAVLMMGRFVEPIDDCPAGNIIGLVGIDQFLLKTGTLTTFEGAHNMKVMKFSVSPVVQVAVEVKNANDLPKLVEGLKRLSKSDPCVLVSMSESGEHIVAGTGELHLEICLQDLENDHAGIPLKISPPVVAYRETVEGESSQTALSKSPNKHNRIYLKAQPIDEEVSLAIEGGKINPRDDFKARARIMADEFGWDVTDARKIWCFGPDGNGPNLVVDQTKAVQYLNEIKDSVVAAFQWATKEGPIFGEQMRSVRVNILDVTLHADAIHRGGGQIIPTMRRATYAGFLLAEPKIQEPVFLVEIQCPEQAIGGIYSVLNKKRGQVVSEEQRPGTPLFTVKAYLPINESFGFTGELRQATGGQAFPQMVFDHWATLGTDPLDPSTKAGEIVLAARKRQGMKEEVPGWQEYYDKL